European Patent Specification EP 3 755 363 B9, published October 4, 2023. Title: PLANTARICIN NC8AB MARKEDLY ENHANCES THE EFFECTS OF ANTIBIOTICS. Applicant: Bengtsson, Torbjorn Khalaf, Hazem. The sequence listing filed with the application follows.

SEQUENCE LISTING (37 sequences)

SEQ ID NO: 1 - protein, 29 aa, Lactobacillus plantarum NC8
DLTTKLWSSWGYYLGKKARWNLKHPYVQF

SEQ ID NO: 2 - protein, 34 aa, Lactobacillus plantarum NC8
SVPTSVYTLGIKILWSAYKHRKTIEKSFNKGFYH

SEQ ID NO: 3 - protein, 14 aa, Lactobacillus plantarum NC8
YTLGIKILWSAYKH

SEQ ID NO: 4 - protein, 15 aa, Lactobacillus plantarum NC8
DLTTKLWSSWGYYLG

SEQ ID NO: 5 - protein, 20 aa, Lactobacillus plantarum NC8
SVPTSVYTLGIKILWSAYKH

SEQ ID NO: 6 - protein, 19 aa, Lactobacillus plantarum NC8
VPTSVYTLGIKILWSAYKH

SEQ ID NO: 7 - protein, 18 aa, Lactobacillus plantarum NC8
PTSVYTLGIKILWSAYKH

SEQ ID NO: 8 - protein, 17 aa, Lactobacillus plantarum NC8
TSVYTLGIKILWSAYKH

SEQ ID NO: 9 - protein, 16 aa, Lactobacillus plantarum NC8
SVYTLGIKILWSAYKH

SEQ ID NO: 10 - protein, 15 aa, Lactobacillus plantarum NC8
VYTLGIKILWSAYKH

SEQ ID NO: 11 - protein, 15 aa, Lactobacillus plantarum NC8
YTLGIKILWSAYKHR

SEQ ID NO: 12 - protein, 16 aa, Lactobacillus plantarum NC8
YTLGIKILWSAYKHRK

SEQ ID NO: 13 - protein, 17 aa, Lactobacillus plantarum NC8
YTLGIKILWSAYKHRKT

SEQ ID NO: 14 - protein, 18 aa, Lactobacillus plantarum NC8
YTLGIKILWSAYKHRKTI

SEQ ID NO: 15 - protein, 19 aa, Lactobacillus plantarum NC8
YTLGIKILWSAYKHRKTIE

SEQ ID NO: 16 - protein, 20 aa, Lactobacillus plantarum NC8
YTLGIKILWSAYKHRKTIEK

SEQ ID NO: 17 - protein, 21 aa, Lactobacillus plantarum NC8
YTLGIKILWSAYKHRKTIEKS

SEQ ID NO: 18 - protein, 22 aa, Lactobacillus plantarum NC8
YTLGIKILWSAYKHRKTIEKSF

SEQ ID NO: 19 - protein, 23 aa, Lactobacillus plantarum NC8
YTLGIKILWSAYKHRKTIEKSFN

SEQ ID NO: 20 - protein, 24 aa, Lactobacillus plantarum NC8
YTLGIKILWSAYKHRKTIEKSFNK

SEQ ID NO: 21 - protein, 25 aa, Lactobacillus plantarum NC8
YTLGIKILWSAYKHRKTIEKSFNKG

SEQ ID NO: 22 - protein, 26 aa, Lactobacillus plantarum NC8
YTLGIKILWSAYKHRKTIEKSFNKGF

SEQ ID NO: 23 - protein, 27 aa, Lactobacillus plantarum NC8
YTLGIKILWSAYKHRKTIEKSFNKGFY

SEQ ID NO: 24 - protein, 28 aa, Lactobacillus plantarum NC8
YTLGIKILWSAYKHRKTIEKSFNKGFYH

SEQ ID NO: 25 - protein, 28 aa, Lactobacillus plantarum NC8
DLTTKLWSSWGYYLGKKARWNLKHPYVQ

SEQ ID NO: 26 - protein, 27 aa, Lactobacillus plantarum NC8
DLTTKLWSSWGYYLGKKARWNLKHPYV

SEQ ID NO: 27 - protein, 26 aa, Lactobacillus plantarum NC8
DLTTKLWSSWGYYLGKKARWNLKHPY

SEQ ID NO: 28 - protein, 25 aa, Lactobacillus plantarum NC8
DLTTKLWSSWGYYLGKKARWNLKHP

SEQ ID NO: 29 - protein, 24 aa, Lactobacillus plantarum NC8
DLTTKLWSSWGYYLGKKARWNLKH

SEQ ID NO: 30 - protein, 23 aa, Lactobacillus plantarum NC8
DLTTKLWSSWGYYLGKKARWNLK

SEQ ID NO: 31 - protein, 22 aa, Lactobacillus plantarum NC8
DLTTKLWSSWGYYLGKKARWNL

SEQ ID NO: 32 - protein, 21 aa, Lactobacillus plantarum NC8
DLTTKLWSSWGYYLGKKARWN

SEQ ID NO: 33 - protein, 20 aa, Lactobacillus plantarum NC8
DLTTKLWSSWGYYLGKKARW

SEQ ID NO: 34 - protein, 19 aa, Lactobacillus plantarum NC8
DLTTKLWSSWGYYLGKKAR

SEQ ID NO: 35 - protein, 18 aa, Lactobacillus plantarum NC8
DLTTKLWSSWGYYLGKKA

SEQ ID NO: 36 - protein, 17 aa, Lactobacillus plantarum NC8
DLTTKLWSSWGYYLGKK

SEQ ID NO: 37 - protein, 16 aa, Lactobacillus plantarum NC8
DLTTKLWSSWGYYLGK